European Patent Application EP 4 353 810 A1, published April 17, 2024. Title: DNA Detection Method and DNA Detection System. Applicant: Hitachi, Ltd. The sequence listing filed with the application follows.

SEQUENCE LISTING (4 sequences)

SEQ ID NO: 1 - DNA, 28 bp, Homo sapiens
gtcacattttcattatttttattataag

SEQ ID NO: 2 - DNA, 22 bp, Homo sapiens
gtatcgtcaaggcactcttgcc

SEQ ID NO: 3 - DNA, 16 bp, Homo sapiens
ttggagctggtggcgt

SEQ ID NO: 4 - DNA, 16 bp, Homo sapiens
ttggagctgctggcgt